European Patent Specification EP 3 549 437 B1, published October 25, 2023. Title: Histidine Engineered Light Chain Antibodies and Genetically Modified Non-Human Animals for Generating the Same. Applicant: Regeneron Pharmaceuticals, Inc. Application to be assigned. The sequence listing filed with the application follows.

SEQUENCE LISTING (146 sequences)

SEQ ID NO: 1 - protein, 95 aa, Artificial
  Synthetic
DIQMTQSPSSLSASVGDRVTITCRASQSISSYLNWYQQKPGKAPKLLIYAASSLQSGVPSRFSGSGSGTDFTLTISSLQPEDFATYYCQQSYSTP

SEQ ID NO: 2 - DNA, 21 bp, Artificial
  Synthetic
  CDS (1)..(21)
cagcagagctacagcaccccc

SEQ ID NO: 3 - protein, 7 aa, Artificial
  Synthetic Construct
QQSYSTP

SEQ ID NO: 4 - DNA, 21 bp, Artificial
  Synthetic
  CDS (1)..(21)
caccatagccacagcacccac

SEQ ID NO: 5 - protein, 7 aa, Artificial
  Synthetic Construct
HHSHSTH

SEQ ID NO: 6 - DNA, 21 bp, Artificial
  Synthetic
  CDS (1)..(21)
caccagagctacagcaccccc

SEQ ID NO: 7 - protein, 7 aa, Artificial
  Synthetic Construct
HQSYSTP

SEQ ID NO: 8 - DNA, 21 bp, Artificial
  Synthetic
  CDS (1)..(21)
cagcatagctacagcaccccc

SEQ ID NO: 9 - protein, 7 aa, Artificial
  Synthetic Construct
QHSYSTP

SEQ ID NO: 10 - DNA, 21 bp, Artificial
  Synthetic
  CDS (1)..(21)
cagcagagccacagcaccccc

SEQ ID NO: 11 - protein, 7 aa, Artificial
  Synthetic Construct
QQSHSTP

SEQ ID NO: 12 - DNA, 21 bp, Artificial
  Synthetic
  CDS (1)..(21)
cagcagagctacagcacccac

SEQ ID NO: 13 - protein, 7 aa, Artificial
  Synthetic Construct
QQSYSTH

SEQ ID NO: 14 - DNA, 21 bp, Artificial
  Synthetic
  CDS (1)..(21)
caccatagctacagcaccccc

SEQ ID NO: 15 - protein, 7 aa, Artificial
  Synthetic Construct
HHSYSTP

SEQ ID NO: 16 - DNA, 21 bp, Artificial
  Synthetic
  CDS (1)..(21)
caccagagccacagcaccccc

SEQ ID NO: 17 - protein, 7 aa, Artificial
  Synthetic Construct
HQSHSTP

SEQ ID NO: 18 - DNA, 21 bp, Artificial
  Synthetic
  CDS (1)..(21)
caccagagctacagcacccac

SEQ ID NO: 19 - protein, 7 aa, Artificial
  Synthetic Construct
HQSYSTH

SEQ ID NO: 20 - DNA, 21 bp, Artificial
  Synthetic
  CDS (1)..(21)
cagcatagccacagcaccccc

SEQ ID NO: 21 - protein, 7 aa, Artificial
  Synthetic Construct
QHSHSTP

SEQ ID NO: 22 - DNA, 21 bp, Artificial
  Synthetic
  CDS (1)..(21)
cagcatagctacagcacccac

SEQ ID NO: 23 - protein, 7 aa, Artificial
  Synthetic Construct
QHSYSTH

SEQ ID NO: 24 - DNA, 21 bp, Artificial
  Synthetic
  CDS (1)..(21)
cagcagagccacagcacccac

SEQ ID NO: 25 - protein, 7 aa, Artificial
  Synthetic Construct
QQSHSTH

SEQ ID NO: 26 - DNA, 21 bp, Artificial
  Synthetic
  CDS (1)..(21)
caccatagccacagcaccccc

SEQ ID NO: 27 - protein, 7 aa, Artificial
  Synthetic Construct
HHSHSTP

SEQ ID NO: 28 - DNA, 21 bp, Artificial
  Synthetic
  CDS (1)..(21)
caccatagctacagcacccac

SEQ ID NO: 29 - protein, 7 aa, Artificial
  Synthetic Construct
HHSYSTH

SEQ ID NO: 30 - DNA, 21 bp, Artificial
  Synthetic
  CDS (1)..(21)
caccagagccacagcacccac

SEQ ID NO: 31 - protein, 7 aa, Artificial
  Synthetic Construct
HQSHSTH

SEQ ID NO: 32 - DNA, 21 bp, Artificial
  Synthetic
  CDS (1)..(21)
cagcatagccacagcacccac

SEQ ID NO: 33 - protein, 7 aa, Artificial
  Synthetic Construct
QHSHSTH

SEQ ID NO: 34 - DNA, 45 bp, Artificial
  Synthetic
cttactactgtcaacatagtcacagtacccatccgatcaccttcg

SEQ ID NO: 35 - DNA, 50 bp, Artificial
  Synthetic
caacttactactgtcaccatagtcacagtacccatccgatcaccttcggc

SEQ ID NO: 36 - DNA, 45 bp, Artificial
  Synthetic
cgaaggtgatcggatgggtactgtgactatgttgacagtagtaag

SEQ ID NO: 37 - DNA, 50 bp, Artificial
  Synthetic
gccgaaggtgatcggatgggtactgtgactatggtgacagtagtaagttg

SEQ ID NO: 38 - DNA, 23 bp, Artificial
  Synthetic
tgggcacaacagacaatcggctg

SEQ ID NO: 39 - DNA, 19 bp, Artificial
  Synthetic
ggtggagaggctattcggc

SEQ ID NO: 40 - DNA, 17 bp, Artificial
  Synthetic
gaacacggcggcatcag

SEQ ID NO: 41 - DNA, 29 bp, Artificial
  Synthetic
ccattatgatgctccatgcctctctgttc

SEQ ID NO: 42 - DNA, 28 bp, Artificial
  Synthetic
aggtgagggtacagataagtgttatgag

SEQ ID NO: 43 - DNA, 27 bp, Artificial
  Synthetic
tgacaaatgccctaattatagtgatca

SEQ ID NO: 44 - DNA, 26 bp, Artificial
  Synthetic
atcagcagaaaccagggaaagcccct

SEQ ID NO: 45 - DNA, 21 bp, Artificial
  Synthetic
gggcaagtcagagcattagca

SEQ ID NO: 46 - DNA, 21 bp, Artificial
  Synthetic
tgcaaactggatgcagcatag

SEQ ID NO: 47 - DNA, 19 bp, Artificial
  Synthetic
ggccacattccatgggttc

SEQ ID NO: 48 - DNA, 20 bp, Artificial
  Synthetic
gcaaacaaaaaccactggcc

SEQ ID NO: 49 - DNA, 37 bp, Artificial
  Synthetic
ctgttcctctaaaactggactccacagtaaatggaaa

SEQ ID NO: 50 - DNA, 22 bp, Artificial
  Synthetic
gggcactggatacgatgtatgg

SEQ ID NO: 51 - DNA, 19 bp, Artificial
  Synthetic
cacagcttgtgcagcctcc

SEQ ID NO: 52 - DNA, 37 bp, Artificial
  Synthetic
agaagaagcctgtactacagcatccgttttacagtca

SEQ ID NO: 53 - DNA, 19 bp, Artificial
  Synthetic
accatagtcacagtaccca

SEQ ID NO: 54 - DNA, 23 bp, Artificial
  Synthetic
agcagtctgcaacctgaagattt

SEQ ID NO: 55 - DNA, 18 bp, Artificial
  Synthetic
cccttggccgaaggtgat

SEQ ID NO: 56 - DNA, 19 bp, Artificial
  Synthetic
atagtcacagtacccatcc

SEQ ID NO: 57 - DNA, 23 bp, Artificial
  Synthetic
agtctgcaacctgaagattttgc

SEQ ID NO: 58 - DNA, 18 bp, Artificial
  Synthetic
cccttggccgaaggtgat

SEQ ID NO: 59 - protein, 108 aa, Artificial
  Synthetic
EIVLTQSPGTLSLSPGERATLSCRASQSVSSSYLAWYQQKPGQAPRLLIYGASSRATGIPDRFSGSGSGTDFTLTISRLEPEDFAVYYCQQYGSSPWTFGQGTKVEIK

SEQ ID NO: 60 - DNA, 54 bp, Artificial
  Synthetic
gattttgcagtgtattactgtcagcagtatggtagctcaccttggacgttcggc

SEQ ID NO: 61 - DNA, 54 bp, Artificial
  Synthetic
gattttgcagtgtattactgtcatcaccatggtcactcaccttggacgttcggc

SEQ ID NO: 62 - DNA, 54 bp, Artificial
  Synthetic
gccgaacgtccaaggtgagtgaccatggtgatgacagtaatacactgcaaaatc

SEQ ID NO: 63 - DNA, 47 bp, Artificial
  Synthetic
gcagtgtattactgtcatcactatggtcactcaccttggacgttcgg

SEQ ID NO: 64 - DNA, 47 bp, Artificial
  Synthetic
ccgaacgtccaaggtgagtgaccatagtgatgacagtaatacactgc

SEQ ID NO: 65 - DNA, 24 bp, Artificial
  Synthetic
aaagagccaccctctcctgcaggg

SEQ ID NO: 66 - DNA, 19 bp, Artificial
  Synthetic
tccaggcaccctgtctttg

SEQ ID NO: 67 - DNA, 26 bp, Artificial
  Synthetic
aagtagctgctgctaacactctgact

SEQ ID NO: 68 - DNA, 15 bp, Artificial
  Synthetic
ctgtcatcaccatgg

SEQ ID NO: 69 - DNA, 23 bp, Artificial
  Synthetic
gcagactggagcctgaagatttt

SEQ ID NO: 70 - DNA, 20 bp, Artificial
  Synthetic
ccgaacgtccaaggtgagtg

SEQ ID NO: 71 - DNA, 17 bp, Artificial
  Synthetic
tactgtcatcactatgg

SEQ ID NO: 72 - DNA, 22 bp, Artificial
  Synthetic
gcagactggagcctgaagattt

SEQ ID NO: 73 - DNA, 20 bp, Artificial
  Synthetic
ccgaacgtccaaggtgagtg

SEQ ID NO: 74 - DNA, 21 bp, Artificial
  Synthetic
  CDS (1)..(21)
cagcagtatggtagctcacct

SEQ ID NO: 75 - protein, 7 aa, Artificial
  Synthetic Construct
QQYGSSP

SEQ ID NO: 76 - DNA, 21 bp, Artificial
  Synthetic
  CDS (1)..(21)
catcaccatggtcactcacct

SEQ ID NO: 77 - protein, 7 aa, Artificial
  Synthetic Construct
HHHGHSP

SEQ ID NO: 78 - DNA, 21 bp, Artificial
  Synthetic
  CDS (1)..(21)
catcactatggtcactcacct

SEQ ID NO: 79 - protein, 7 aa, Artificial
  Synthetic Construct
HHYGHSP

SEQ ID NO: 80 - protein, 108 aa, Artificial
  Synthetic
DIQMTQSPSSLSASVGDRVTITCRASQSISSYLNWYQQKPGKAPKLLIYAASSLQSGVPSRFSGSGSGTDFTLTISSLQPEDFATYYCQQSYSTPPITFGQGTRLEIK

SEQ ID NO: 81 - DNA, 50 bp, Artificial
  Synthetic
caacttactactgtcaacagagttacagtacccctccgatcaccttcggc

SEQ ID NO: 82 - DNA, 9652 bp, Artificial
  synthetic
gcaccacttcgtcgcagcgcaggctttggtctcccttgtccgtgcggcgcacgcccaccgagtttacgcaccagcacaccgaggtctggttggtaccgaagttcctattccgaagttcctattctctagaaagtataggaacttctcgcgcgtctggcctccgaggcctccgcgccgggttttggcgcctcccgcgggcgcccccctcctcacggcgagcgctgccacgtcagacgaagggcgcagcgagcgtcctgatccttccgcccggacgctcaggacagcggcccgctgctcataagactcggccttagaaccccagtatcagcagaaggacattttaggacgggacttgggtgactctagggcactggttttctttccagagagcggaacaggcgaggaaaagtagtcccttctcggcgattctgcggagggatctccgtggggcggtgaacgccgatgattatataaggacgcgccgggtgtggcacagctagttccgtcgcagccgggatttgggtcgcggttcttgtttgtggatcgctgtgatcgtcacttggtgagtagcgggctgctgggctggccggggctttcgtggccgccgggccgctcggtgggacggaagcgtgtggagagaccgccaagggctgtagtctgggtccgcgagcaaggttgccctgaactgggggttggggggagcgcagcaaaatggcggctgttcccgagtcttgaatggaagacgcttgtgaggcgggctgtgaggtcgttgaaacaaggtggggggcatggtgggcggcaagaacccaaggtcttgaggccttcgctaatgcgggaaagctcttattcgggtgagatgggctggggcaccatctggggaccctgacgtgaagtttgtcactgactggagaactcggtttgtcgtctgttgcgggggcggcagttatggcggtgccgttgggcagtgcacccgtacctttgggagcgcgcgccctcgtcgtgtcgtgacgtcacccgttctgttggcttataatgcagggtggggccacctgccggtaggtgtgcggtaggcttttctccgtcgcaggacgcagggttcgggcctagggtaggctctcctgaatcgacaggcgccggacctctggtgaggggagggataagtgaggcgtcagtttctttggtcggttttatgtacctatcttcttaagtagctgaagctccggttttgaactatgcgctcggggttggcgagtgtgttttgtgaagttttttaggcaccttttgaaatgtaatcatttgggtcaatatgtaattttcagtgttagactagtaaattgtccgctaaattctggccgtttttggcttttttgttagacgtcgagctctagattgggaacccgggtctctcgaattgttgacaattaatcatcggcatagtatatcggcatagtataatacgacaaggtgaggaactaaaccatccaccatgattgaacaagatggattgcacgcaggttctccggccgcttgggtggagaggctattcggctatgactgggcacaacagacaatcggctgctctgatgccgccgtgttccggctgtcagcgcaggggcgcccggttctttttgtcaagaccgacctgtccggtgccctgaatgaactgcaggacgaggcagcgcggctatcgtggctggccacgacgggcgttccttgcgcagctgtgctcgacgttgtcactgaagcgggaagggactggctgctattgggcgaagtgccggggcaggatctcctgtcatctcaccttgctcctgccgagaaagtatccatcatggctgatgcaatgcggcggctgcatacgcttgatccggctacctgcccattcgaccaccaagcgaaacatcgcatcgagcgagcacgtactcggatggaagccggtcttgtcgatcaggatgatctggacgaagagcatcaggggctcgcgccagccgaactgttcgccaggctcaaggcgcgcatgcccgacggcgaggatctcgtcgtgacccatggcgatgcctgcttgccgaatatcatggtggaaaatggccgcttttctggattcatcgactgtggccggctgggtgtggcggaccgctatcaggacatagcgttggctacccgtgatattgctgaagagcttggcggcgaatgggctgaccgcttcctcgtgctttacggtatcgccgctcccgattcgcagcgcatcgccttctatcgccttcttgacgagttcttctgaagatccgctgtaagtctgcagaaattgatgatctattaaacaataaagatgtccactaaaatggaagtttttcctgtcatactttgttaagaagggtgagaacagagtacctacattttgaatggaaggattggagctacgggggtgggggtggggtgggattagataaatgcctgctctttactgaaggctctttactattgctttatgataatgtttcatagttggatatcataatttaaacaagcaaaaccaaattaagggccagctcattcctcccactcatgatctatagatctatagatctctcgtgggatcattgtttttctcttgattcccactttgtggttctaagtactgtggtttccaaatgtgtcagtttcatagcctgaagaacgagatcagcagcctctgttccacatacacttcattctcagtattgttttgccaagttctaattccatcagacctcgacctgcagcccctagagaagttcctattccgaagttcctattctctagaaagtataggaacttcctagggtttcaccggtggcgcgccgagagaggaaagagagcagcgataccgaaaatgtcctcagcgagaagctaccacagaggatgaatggagatcaagcccacgtggaaacatgggaaaatgtctcagtatttttccacctaagaagggagggagatggggtatgtatacacctccctgtcctcactgattgagggctttccgagaggatgctcattccaggtgctgtgataggccatgtgtacaggcagggctgccttctccagcttcagatagagcagtgaggaaaagatatggccatggggggtcagcagaagtacagcaaagggaaaagggaaagggtagcaagagtgacaactatattcaccccccccacacacacacacacacacacgaaattgtgtattgcaatccagaactgcttctctctgaacctaaatcttagcaagcagtttaccagtaactgcccttgaaattcaggcccctggaaaggagcagggggttgtgtacaggctataccacagcagtctgcccacccttagtgatgcatgagtaatgctccctggactccccaggttctagtcttctcatgtcgatgtagttgattccacttcccttgctgcacaaccaggctgggatgcctgggcagaggcagacatgtgaggtataggggttcaaatctgtttccaagttttatccagcttcaaagcatttctccgtgtacatgagcggtggcttgacaggagatggagactctctttcctggatgtgaggcaaggaggcaggcgtctgagtcaggatgatgtccctactcactgctaaagagaaaagtggctttgatggtgcagggcagggaaatgcactgagtggtcgccaccctcacagaagagaaagtgttcactgacctggcctttccccagggcctctccctcccattgctttccagaaagccatgatttttgagagccacacctgaacactcacaaacattatggtgggaaaagcagatcagagcattaggcaagttgcattaccttggccttcttcctttggagacaattgatgtggggttctagattgacccagagtttcaagtttatcctgattcaggcttcaacagctggaggaagaaacagagatgttttttgaagtaaacagatctagcattactaatcaacccttcatactgatgacctatgggaaataatacccaagggcagaaaaatgggcagaataaggggagccccaaaccaagacgaagctgctgcccattgagaccctgggtattacagagacctatagctctggataatggaagatctatgagtggcacaggcgctgaggaatcacagcatcattatcgtgcatctgcagggaattgcttgtaaatatactggtaattacaaatgtttaaggtcactacaaatactttggagtgtattaaatatgcttctgataaagactgtttttctcacatgaaacaatgggaaccatgtgacaatcacagaggtgttgttactatagcaaaagggattgttactctccacatccctttaagtaacttgaaggcctgatagacccaccctctaagacttcattagacattccctacgaatggttatactctcctgtatactcccaatacaactctaaaatatattattccatatagtccttaggtttgtattaaagtttgacttttttccttcaaaatatctcttgtcacaacagcggctctagagagaaatacattccctccaggcaaatctatgctgcgctggtctgacctgggaccctggggacattgcccctgtgctgagttactaagatgagccagccctgcagctgtgctcagcctgccccatgccctgctgattgatttgcatgttccagagcacagccccctgccctgaagacttttttatgggctggtcgcaccctgtgcaggagtcagtctcagtcaggacacagcatggacatgagggtccccgctcagctcctggggctcctgctactctggctccgaggtaaggatggagaacactaggaatttactcagccagtgtgctcagtactgactggaacttcagggaagttctctgataacatgattaatagtaagaatatttgtttttatgtttccaatctcaggtgccagatgtgacatccagatgacccagtctccatcctccctgtctgcatctgtaggagacagagtcaccatcacttgccgggcaagtcagagcattagcagctatttaaattggtatcagcagaaaccagggaaagcccctaagctcctgatctatgctgcatccagtttgcaaagtggggtcccatcaaggttcagtggcagtggatctgggacagatttcactctcaccatcagcagtctgcaacctgaagattttgcaacttactactgtcaacagagttacagtacccctcccacagtgttacaagtcataacataaacctccaaggaagcagatgtgtgaggacgagccaccccagatgctcctcctggtgcctccatctgctgagagcatttctcaaactcagtcaggttttgaaagtcattgggagacttttgtagaggggaccagggaggctcctctgaactctaagcctcttttgccccggatccgatcaggaaaatagcaaccgagtgactggactattaaagcatcccctctgtggagaaaaggactatggcaacagcttgccacctataagagacaaatatgtcactcagctggatgctgggtctaccatgaccacccttgagatgaacttatgccatgtttttggatgcccactgagactttgctttgaccaaggaaagttctttactgcccaaatgacgtcaatggacacactctcatgggacatgatggattttccatacaccttgttatccaaaggccaatggatctatttaatgctagaacagctgactcacacggcaactgaagagtgtacatcagggcaacctgctagtagagtggtaccccatctgactacagcaattggacattaaacactgcactgcagagcaagggaaagacggcacggaggtgcaggttgaaaaacactgagttgagtgaggaagaagttgggcaaggccagtttcctgatagagctgccactgtgaaatcccaaactcagtgtttccaatcatttttttccttttatagtgatgttcttgggggtgttgcagtttaggccaccatgataacccagacaggcctcctaactctaattggatggaatgattcccctgggtgccttctatgggttccacaggatcaagaaatatcagggtgttaatttccttctgctggtaggagggtcatctgattcctccattagggtggatgacgttatcagacatgtcaattttctacagtacttgacctgccttctagaactggacaaccgagggtgaaaggactggatcaagcaacaatggcaatgggtgcccaaagaggtagtagtctcagaacagggagagacagactgagtccctccactaactcagcccaacacctgtggatgagtaggggatgcctgagatcctggggtggatgggaggtggggcactgatctgtcaatctgctttttcttcaaggatcaggcagcagagacccagaagcttcatgtctttgtaaggctcttccaagccaacacagataatttgacaaaacactgtatctgcatcccagacctcaccctgtcacagactgaagtggttgtttcatcctactaagggtaaactataccagctatacagaataaaaagactggatagtttagaggatcacccaagaaatagttctttgcctgcatggacaaaaccatcttctgtctttagggaaatggtatcactaccctgaggatttggagcccaggtctcacttatctgtgcagttgtgaaagtcctcacacccacagtgctgaggttaattgaatgttactcttttaatttctgcaaagaatgagacagcttctggaccctcaggaaagatcactaacaagtaaatacaagtatatccggaagataaagttgtaatagactcttcctttcaacctgatccatcatgcatttagggagctgactgggcacaagttggagcagaaagagaaaaatgaaaccacagccttctattttgtttctaacagacttgtaccaaacattctgtggctcaatctaggtgatggtgagacaagaggacacaggggttaaattctgtggccgcaggggagaagttctaccctcagactgagccaacggccttttctggcctgatcacctgggcatgggctgctgagagcagaaaggggaggcagattgtctctgcagctgcaagcccagcacccgccccagctgctttgcatgtccctcccagccgccctgcagtccagagcccatatcaatgcctgggtcagagctctggagaagagctgctcagttaggacccagagggaaccatggaaaccccagcgcagcttctcttcctcctgctactctggctcccaggtgaggggaacatgggatggttttgcatgtcagtgaaaaccctctcaagtcctgttacctggcaactctgctcagtcaatacaataattaaagctcaatataaagcaataattctggctcttctgggaagacaatgggtttgatttagattacatgggtgacttttctgttttatttccaatctcagataccaccggagaaattgtgttgacgcagtctccaggcaccctgtctttgtctccaggggaaagagccaccctctcctgcagggccagtcagagtgttagcagcagctacttagcctggtaccagcagaaacctggccaggctcccaggctcctcatctatggtgcatccagcagggccactggcatcccagacaggttcagtggcagtgggtctgggacagacttcactctcaccatcagcagactggagcctgaagattttgcagtgtattactgtcagcagtatggtagctcacctcccacagtgattcagcttgaaacaaaaacctctgcaagaccttcattgtttactagattataccagctgcttcctttacagatagctgctgcaatgacaactcaattttagcatctcttctctgcttgggcattttggggatcttaaaaaagtaatcccttgatatatttttgactctgattcctgcatttttcctcagaccaagatggacagccaggtttaagcacagtttcacagtaatggccactggatcagatttacatcagtggatgtcagtaaaggtcccaaccagagccataaggcaacaacaatagcaacaaataatcaaaattggaaaagaagaattaaagctgtcataattcactgatgaaggattgtgtgcagataaaattcaaatttgtctacagagaaactactaaaattgacatgagaaatagaaaatcattagattcaagatcaatttattaattcatagattcaaaaatcaatttcatttctgcataataaaaaatgctaaaaattaacattataaaacaaacacaccatttacaaaaacatcaaagtatcaattatttaaaaaaaatagactaaatacactgacgtctccagaatattattttgaaaaataaaagaaaacctaagtaaatagaaattcagttcaaagactgaatgtctcagtactataaaaatgtcaattcttcaaagattaaaatattgattacatataagaaaaatcaaaatcctaaagtatactccaatttaaattaagaagctaatctaaatattatatgggaatgtcaaggatgtagaatagccacagtgaacctgaagaaacaccaaaatgagaacttccagtgcctgaatacctggaatatagtgtgggtggcagtatggtgatggtgagatcagaagtttaaaaatttgcaaacgtgcttatttttggaaataatcactacgcagatgtagccaaaccctcttcaactgtggcgtacgctcaggtcaattccaaagagtaccagattctttcaaaaagtcagatgagtaagggatagaaaattagttcatcttaaggaacagccaagcgctagccagttaagtgaggcatctcaattgcaagattttctctgcatcggtcaggttagtgatattaacagcgaaaagagatttttgttaaggggaaagtaattaagttaacactgtggatcaccttcggccaagggacacgactggagattaaacgtaagtaatttttcactattgtcttctgaaatttgggtctgatggccagtattgacttttagaggcttaaataggagtttggtaaagattggtaaatgagggcatttaagatttgccatgggttgcaaaagttaaactcagcttcaaaaatggatttggagaaaaaaagattaaattgctctaaactgaatgacacaaagtaaaaaaaaaaagtgtaactaaaaaggaacccttgtatttctaaggagcaaaagtaaatttatttttgttcactcttgccaaatattgtattggttgttgctgattatgcatgatacagaaaagtggaaaaatacattttttagtctttctcccttttgtttgataaattattttgtcagacaacaataaaaatcaatagcacgccctaagatctagatgcatgctcgagtgccatttcattacctctttctccgcacccgacatagataagcttatcgataccgtcgacctcgagggggggcccggtaccccgtggcatacagtgtcagattttctgtttatcaagctagtgagattaggggcaaaaa

SEQ ID NO: 83 - DNA, 10867 bp, Artificial
  Synthetic
gcaccacttcgtcgcagcgcaggctttggtctcccttgtccgtgcggcgcacgcccaccgagtttacgcaccagcacaccgaggtctggttggtaccgaagttcctattccgaagttcctattctctagaaagtataggaacttctcgcgcgtctggcctccgaggcctccgcgccgggttttggcgcctcccgcgggcgcccccctcctcacggcgagcgctgccacgtcagacgaagggcgcagcgagcgtcctgatccttccgcccggacgctcaggacagcggcccgctgctcataagactcggccttagaaccccagtatcagcagaaggacattttaggacgggacttgggtgactctagggcactggttttctttccagagagcggaacaggcgaggaaaagtagtcccttctcggcgattctgcggagggatctccgtggggcggtgaacgccgatgattatataaggacgcgccgggtgtggcacagctagttccgtcgcagccgggatttgggtcgcggttcttgtttgtggatcgctgtgatcgtcacttggtgagtagcgggctgctgggctggccggggctttcgtggccgccgggccgctcggtgggacggaagcgtgtggagagaccgccaagggctgtagtctgggtccgcgagcaaggttgccctgaactgggggttggggggagcgcagcaaaatggcggctgttcccgagtcttgaatggaagacgcttgtgaggcgggctgtgaggtcgttgaaacaaggtggggggcatggtgggcggcaagaacccaaggtcttgaggccttcgctaatgcgggaaagctcttattcgggtgagatgggctggggcaccatctggggaccctgacgtgaagtttgtcactgactggagaactcggtttgtcgtctgttgcgggggcggcagttatggcggtgccgttgggcagtgcacccgtacctttgggagcgcgcgccctcgtcgtgtcgtgacgtcacccgttctgttggcttataatgcagggtggggccacctgccggtaggtgtgcggtaggcttttctccgtcgcaggacgcagggttcgggcctagggtaggctctcctgaatcgacaggcgccggacctctggtgaggggagggataagtgaggcgtcagtttctttggtcggttttatgtacctatcttcttaagtagctgaagctccggttttgaactatgcgctcggggttggcgagtgtgttttgtgaagttttttaggcaccttttgaaatgtaatcatttgggtcaatatgtaattttcagtgttagactagtaaattgtccgctaaattctggccgtttttggcttttttgttagacgtcgagctctagattgggaacccgggtctctcgaattgttgacaattaatcatcggcatagtatatcggcatagtataatacgacaaggtgaggaactaaaccatccaccatgattgaacaagatggattgcacgcaggttctccggccgcttgggtggagaggctattcggctatgactgggcacaacagacaatcggctgctctgatgccgccgtgttccggctgtcagcgcaggggcgcccggttctttttgtcaagaccgacctgtccggtgccctgaatgaactgcaggacgaggcagcgcggctatcgtggctggccacgacgggcgttccttgcgcagctgtgctcgacgttgtcactgaagcgggaagggactggctgctattgggcgaagtgccggggcaggatctcctgtcatctcaccttgctcctgccgagaaagtatccatcatggctgatgcaatgcggcggctgcatacgcttgatccggctacctgcccattcgaccaccaagcgaaacatcgcatcgagcgagcacgtactcggatggaagccggtcttgtcgatcaggatgatctggacgaagagcatcaggggctcgcgccagccgaactgttcgccaggctcaaggcgcgcatgcccgacggcgaggatctcgtcgtgacccatggcgatgcctgcttgccgaatatcatggtggaaaatggccgcttttctggattcatcgactgtggccggctgggtgtggcggaccgctatcaggacatagcgttggctacccgtgatattgctgaagagcttggcggcgaatgggctgaccgcttcctcgtgctttacggtatcgccgctcccgattcgcagcgcatcgccttctatcgccttcttgacgagttcttctgaagatccgctgtaagtctgcagaaattgatgatctattaaacaataaagatgtccactaaaatggaagtttttcctgtcatactttgttaagaagggtgagaacagagtacctacattttgaatggaaggattggagctacgggggtgggggtggggtgggattagataaatgcctgctctttactgaaggctctttactattgctttatgataatgtttcatagttggatatcataatttaaacaagcaaaaccaaattaagggccagctcattcctcccactcatgatctatagatctatagatctctcgtgggatcattgtttttctcttgattcccactttgtggttctaagtactgtggtttccaaatgtgtcagtttcatagcctgaagaacgagatcagcagcctctgttccacatacacttcattctcagtattgttttgccaagttctaattccatcagacctcgacctgcagcccctagagaagttcctattccgaagttcctattctctagaaagtataggaacttcctagggtttcaccggtggcgcgccgagagaggaaagagagcagcgataccgaaaatgtcctcagcgagaagctaccacagaggatgaatggagatcaagcccacgtggaaacatgggaaaatgtctcagtatttttccacctaagaagggagggagatggggtatgtatacacctccctgtcctcactgattgagggctttccgagaggatgctcattccaggtgctgtgataggccatgtgtacaggcagggctgccttctccagcttcagatagagcagtgaggaaaagatatggccatggggggtcagcagaagtacagcaaagggaaaagggaaagggtagcaagagtgacaactatattcaccccccccacacacacacacacacacacgaaattgtgtattgcaatccagaactgcttctctctgaacctaaatcttagcaagcagtttaccagtaactgcccttgaaattcaggcccctggaaaggagcagggggttgtgtacaggctataccacagcagtctgcccacccttagtgatgcatgagtaatgctccctggactccccaggttctagtcttctcatgtcgatgtagttgattccacttcccttgctgcacaaccaggctgggatgcctgggcagaggcagacatgtgaggtataggggttcaaatctgtttccaagttttatccagcttcaaagcatttctccgtgtacatgagcggtggcttgacaggagatggagactctctttcctggatgtgaggcaaggaggcaggcgtctgagtcaggatgatgtccctactcactgctaaagagaaaagtggctttgatggtgcagggcagggaaatgcactgagtggtcgccaccctcacagaagagaaagtgttcactgacctggcctttccccagggcctctccctcccattgctttccagaaagccatgatttttgagagccacacctgaacactcacaaacattatggtgggaaaagcagatcagagcattaggcaagttgcattaccttggccttcttcctttggagacaattgatgtggggttctagattgacccagagtttcaagtttatcctgattcaggcttcaacagctggaggaagaaacagagatgttttttgaagtaaacagatctagcattactaatcaacccttcatactgatgacctatgggaaataatacccaagggcagaaaaatgggcagaataaggggagccccaaaccaagacgaagctgctgcccattgagaccctgggtattacagagacctatagctctggataatggaagatctatgagtggcacaggcgctgaggaatcacagcatcattatcgtgcatctgcagggaattgcttgtaaatatactggtaattacaaatgtttaaggtcactacaaatactttggagtgtattaaatatgcttctgataaagactgtttttctcacatgaaacaatgggaaccatgtgacaatcacagaggtgttgttactatagcaaaagggattgttactctccacatccctttaagtaacttgaaggcctgatagacccaccctctaagacttcattagacattccctacgaatggttatactctcctgtatactcccaatacaactctaaaatatattattccatatagtccttaggtttgtattaaagtttgacttttttccttcaaaatatctcttgtcacaacagcggctctagagagaaatacattccctccaggcaaatctatgctgcgctggtctgacctgggaccctggggacattgcccctgtgctgagttactaagatgagccagccctgcagctgtgctcagcctgccccatgccctgctgattgatttgcatgttccagagcacagccccctgccctgaagacttttttatgggctggtcgcaccctgtgcaggagtcagtctcagtcaggacacagcatggacatgagggtccccgctcagctcctggggctcctgctactctggctccgaggtaaggatggagaacactaggaatttactcagccagtgtgctcagtactgactggaacttcagggaagttctctgataacatgattaatagtaagaatatttgtttttatgtttccaatctcaggtgccagatgtgacatccagatgacccagtctccatcctccctgtctgcatctgtaggagacagagtcaccatcacttgccgggcaagtcagagcattagcagctatttaaattggtatcagcagaaaccagggaaagcccctaagctcctgatctatgctgcatccagtttgcaaagtggggtcccatcaaggttcagtggcagtggatctgggacagatttcactctcaccatcagcagtctgcaacctgaagattttgcaacttactactgtcaacagagttacagtacccctcccacagtgttacaagtcataacataaacctccaaggaagcagatgtgtgaggacgagccaccccagatgctcctcctggtgcctccatctgctgagagcatttctcaaactcagtcaggttttgaaagtcattgggagacttttgtagaggggaccagggaggctcctctgaactctaagcctcttttgccccggatccgatcaggaaaatagcaaccgagtgactggactattaaagcatcccctctgtggagaaaaggactatggcaacagcttgccacctataagagacaaatatgtcactcagctggatgctgggtctaccatgaccacccttgagatgaacttatgccatgtttttggatgcccactgagactttgctttgaccaaggaaagttctttactgcccaaatgacgtcaatggacacactctcatgggacatgatggattttccatacaccttgttatccaaaggccaatggatctatttaatgctagaacagctgactcacacggcaactgaagagtgtacatcagggcaacctgctagtagagtggtaccccatctgactacagcaattggacattaaacactgcactgcagagcaagggaaagacggcacggaggtgcaggttgaaaaacactgagttgagtgaggaagaagttgggcaaggccagtttcctgatagagctgccactgtgaaatcccaaactcagtgtttccaatcatttttttccttttatagtgatgttcttgggggtgttgcagtttaggccaccatgataacccagacaggcctcctaactctaattggatggaatgattcccctgggtgccttctatgggttccacaggatcaagaaatatcagggtgttaatttccttctgctggtaggagggtcatctgattcctccattagggtggatgacgttatcagacatgtcaattttctacagtacttgacctgccttctagaactggacaaccgagggtgaaaggactggatcaagcaacaatggcaatgggtgcccaaagaggtagtagtctcagaacagggagagacagactgagtccctccactaactcagcccaacacctgtggatgagtaggggatgcctgagatcctggggtggatgggaggtggggcactgatctgtcaatctgctttttcttcaaggatcaggcagcagagacccagaagcttcatgtctttgtaaggctcttccaagccaacacagataatttgacaaaacactgtatctgcatcccagacctcaccctgtcacagactgaagtggttgtttcatcctactaagggtaaactataccagctatacagaataaaaagactggatagtttagaggatcacccaagaaatagttctttgcctgcatggacaaaaccatcttctgtctttagggaaatggtatcactaccctgaggatttggagcccaggtctcacttatctgtgcagttgtgaaagtcctcacacccacagtgctgaggttaattgaatgttactcttttaatttctgcaaagaatgagacagcttctggaccctcaggaaagatcactaacaagtaaatacaagtatatccggaagataaagttgtaatagactcttcctttcaacctgatccatcatgcatttagggagctgactgggcacaagttggagcagaaagagaaaaatgaaaccacagccttctattttgtttctaacagacttgtaccaaacattctgtggctcaatctaggtgatggtgagacaagaggacacaggggttaaattctgtggccgcaggggagaagttctaccctcagactgagccaacggccttttctggcctgatcacctgggcatgggctgctgagagcagaaaggggaggcagattgtctctgcagctgcaagcccagcacccgccccagctgctttgcatgtccctcccagccgccctgcagtccagagcccatatcaatgcctgggtcagagctctggagaagagctgctcagttaggacccagagggaaccatggaaaccccagcgcagcttctcttcctcctgctactctggctcccaggtgaggggaacatgggatggttttgcatgtcagtgaaaaccctctcaagtcctgttacctggcaactctgctcagtcaatacaataattaaagctcaatataaagcaataattctggctcttctgggaagacaatgggtttgatttagattacatgggtgacttttctgttttatttccaatctcagataccaccggagaaattgtgttgacgcagtctccaggcaccctgtctttgtctccaggggaaagagccaccctctcctgcagggccagtcagagtgttagcagcagctacttagcctggtaccagcagaaacctggccaggctcccaggctcctcatctatggtgcatccagcagggccactggcatcccagacaggttcagtggcagtgggtctgggacagacttcactctcaccatcagcagactggagcctgaagattttgcagtgtattactgtcagcagtatggtagctcacctcccacagtgattcagcttgaaacaaaaacctctgcaagaccttcattgtttactagattataccagctgcttcctttacagatagctgctgcaatgacaactcaattttagcatctcttctctgcttgggcattttggggatcttaaaaaagtaatcccttgatatatttttgactctgattcctgcatttttcctcagaccaagatggacagccaggtttaagcacagtttcacagtaatggccactggatcagatttacatcagtggatgtcagtaaaggtcccaaccagagccataaggcaacaacaatagcaacaaataatcaaaattggaaaagaagaattaaagctgtcataattcactgatgaaggattgtgtgcagataaaattcaaatttgtctacagagaaactactaaaattgacatgagaaatagaaaatcattagattcaagatcaatttattaattcatagattcaaaaatcaatttcatttctgcataataaaaaatgctaaaaattaacattataaaacaaacacaccatttacaaaaacatcaaagtatcaattatttaaaaaaaatagactaaatacactgacgtctccagaatattattttgaaaaataaaagaaaacctaagtaaatagaaattcagttcaaagactgaatgtctcagtactataaaaatgtcaattcttcaaagattaaaatattgattacatataagaaaaatcaaaatcctaaagtatactccaatttaaattaagaagctaatctaaatattatatgggaatgtcaaggatgtagaatagccacagtgaacctgaagaaacaccaaaatgagaacttccagtgcctgaatacctggaatatagtgtgggtggcagtatggtgatggtgagatcagaagtttaaaaatttgcaaacgtgcttatttttggaaataatcactacgcagatgtagccaaaccctcttcaactgtggcgtacgcacctgctcgaaaagggagttgagcttcagcagctgacccaggactctgttcccctttggtgagaagggtttttgttcagcaagacaatggagagctctcactgtggtggacgttcggccaagggaccaaggtggaaatcaaacgtgagtagaatttaaactttgcttcctcagttgtctgtgtcttctgttccctgtgtctatgaagtgatctataagctgactctgcaatcagcctctgatatccttcagggaaaagataaagataagtctgtagtcaaactcgagaattgattgcacattttctttgaagagcaagcaagattcagtcattgggtgagaataacttgtctaagtaatagcttcagaaatgtcctggggaacataacatgttctggacagagccttggtcaattgtcagaaagggagtttttgtataggagggaagttaagaggaaccattgtgtgtacacttttggccaggggaccaagctggagatcaaacgtaagtacttttttccactgattcttcactgttgctaattagtttactttgtgttcctttgtgtggattttcattagtcggatgccagggatctaacaaacttcattcccaggttaggtacagaggaggggaaattgttccacaggaagctagcttgtggctaatttttaagatttctaaatcaaaataacttcattgggggaaagaggcttgctgagctttcagggaggtttttgtaaagggaaaagttaagacgaatcactgtgattcactttcggccctgggaccaaagtggatatcaaacgtaagtacatctgtctcaattattcgtgagattttagtgccattgtatcatttgtgcaagttttgtgatattttggttgaataaacctggtgacccagaagtaaatagcaggacaccagaaaatgaacttaaaaagctgagcaaatagacgaatcattgggtttgagaggagaataggattcatgggggaaatggggaagaaatagctagatttttctctgaacaagcagcctatctcatatgattggcttcaagagaggtttttgttgaggggaaagggtgagatccctcactgtggctcactttcggcggagggaccaaggtggagatcaaacgtaagtgcactttcctaatgctttttcttataaggttttaaatttggagcgtttttgtgtttgagatattagctcaggtcaattccaaagagtaccagattctttcaaaaagtcagatgagtaagggatagaaaattagttcatcttaaggaacagccaagcgctagccagttaagtgaggcatctcaattgcaagattttctctgcatcggtcaggttagtgatattaacagcgaaaagagatttttgttaaggggaaagtaattaagttaacactgtggatcaccttcggccaagggacacgactggagattaaacgtaagtaatttttcactattgtcttctgaaatttgggtctgatggccagtattgacttttagaggcttaaataggagtttggtaaagattggtaaatgagggcatttaagatttgccatgggttgcaaaagttaaactcagcttcaaaaatggatttggagaaaaaaagattaaattgctctaaactgaatgacacaaagtaaaaaaaaaagtgtaactaaaaaggaacccttgtatttctaaggagcaaaagtaaatttatttttgttcactcttgccaaatattgtattggttgttgctgattatgcatgatacagaaaagtggaaaaatacattttttagtctttctcccttttgtttgataaattattttgtcagacaactataaaaatcaatagcacgccctaagatctagatgcatgctcgagtgccatttcattacctctttctccgcacccgacatagataaagcttatcgataccgtcgacctcgagggggggcccggtaccacgtggcatacagtgtcagattttctgtttatcaagctagtgagattaggggcaaaa

SEQ ID NO: 84 - DNA, 23 bp, Artificial
  Synthetic
tcttttgccccggatccgatcag

SEQ ID NO: 85 - DNA, 23 bp, Artificial
  Synthetic
gggaggctcctctgaactctaag

SEQ ID NO: 86 - DNA, 21 bp, Artificial
  Synthetic
gtccagtcactcggttgctat

SEQ ID NO: 87 - DNA, 22 bp, Artificial
  Synthetic
cttcaactgtggcgtacgcacc

SEQ ID NO: 88 - DNA, 21 bp, Artificial
  Synthetic
acgcagatgtagccaaaccct

SEQ ID NO: 89 - DNA, 20 bp, Artificial
  Synthetic
cagctgctgaagctcaactc

SEQ ID NO: 90 - DNA, 22 bp, Artificial
  Synthetic
aagaagcacacgactgaggcac

SEQ ID NO: 91 - DNA, 24 bp, Artificial
  Synthetic
ctcactggatggtgggaagatgga

SEQ ID NO: 92 - DNA, 16 bp, Artificial
  Synthetic
gtaaaacgacggccag

SEQ ID NO: 93 - DNA, 17 bp, Artificial
  Synthetic
caggaaacagctatgac

SEQ ID NO: 94 - protein, 39 aa, Artificial
  Synthetic
QPEDFATYYCQQSYSTPYTFGQGTKLEIKRADAAPTVSI

SEQ ID NO: 95 - protein, 39 aa, Artificial
  Synthetic
QPEDFATYYCQQSYSTPFTFGPGTKVDIKRADAAPTVSI

SEQ ID NO: 96 - protein, 39 aa, Artificial
  Synthetic
EPEDFAVYYCQQYGSSPRTFGQGTKVEIKRADAAPTVSI

SEQ ID NO: 97 - protein, 38 aa, Artificial
  Synthetic
EPEDFAVYYCQQYGSSRTFGQGTKVEIKRADAAPTVSI

SEQ ID NO: 98 - protein, 39 aa, Artificial
  Synthetic
EPEDFAVYYCQQYGSSPWTFGQGTKVEIKRADAAPTVSI

SEQ ID NO: 99 - protein, 39 aa, Artificial
  Synthetic
DPEDFAVYYCQQYGSSPRTFGQGTKVEIKRADAAPTVSI

SEQ ID NO: 100 - protein, 39 aa, Artificial; identical to SEQ ID NO: 96
  Synthetic

SEQ ID NO: 101 - protein, 39 aa, Artificial; identical to SEQ ID NO: 98
  Synthetic

SEQ ID NO: 102 - protein, 39 aa, Artificial
  Synthetic
EPEDFAVYYCQQYGSSPPTFGQGTKVEIKRADAAPTVSI

SEQ ID NO: 103 - protein, 39 aa, Artificial
  Synthetic
EPEDFAVYYCQQYGSSPYTFGQGTKLEIKRADAAPTVSI

SEQ ID NO: 104 - protein, 39 aa, Artificial
  Synthetic
EPEDFAVYYCQQYGSSIFTFGPGTKVDIKRADAAPTVSI

SEQ ID NO: 105 - DNA, 51 bp, Artificial
  Synthetic
caacttactactgtcaacagagttacagtacccctcccacagtgttacaag

SEQ ID NO: 106 - DNA, 51 bp, Artificial
  Synthetic
caacttactactgtcaccatagtcacagtacccatcccacagtgttacaag

SEQ ID NO: 107 - DNA, 51 bp, Artificial
  Synthetic
cttgtaacactgtgggatgggtactgtgactatggtgacagtagtaagttg

SEQ ID NO: 108 - DNA, 41 bp, Artificial
  Synthetic
gcagtgtattactgtcagcagtatggtagctcacctcccac

SEQ ID NO: 109 - DNA, 60 bp, Artificial
  Synthetic
agattttgcagtgtattactgtcaccatcatggtcactcacctcccacagtgattcagct

SEQ ID NO: 110 - DNA, 60 bp, Artificial; identical to SEQ ID NO: 109
  Synthetic

SEQ ID NO: 111 - DNA, 18 bp, Artificial
  Synthetic
aacttactactgtcacca

SEQ ID NO: 112 - DNA, 19 bp, Artificial
  Synthetic
cagcagtctgcaacctgaa

SEQ ID NO: 113 - DNA, 18 bp, Artificial
  Synthetic
ggctcgtcctcacacatc

SEQ ID NO: 114 - DNA, 17 bp, Artificial
  Synthetic
ttactgtcaccatcatg

SEQ ID NO: 115 - DNA, 19 bp, Artificial
  Synthetic
gcagactggagcctgaaga

SEQ ID NO: 116 - DNA, 23 bp, Artificial
  Synthetic
aagctgaatcactgtgggaggtg

SEQ ID NO: 117 - DNA, 51 bp, Artificial; identical to SEQ ID NO: 105
  Synthetic

SEQ ID NO: 118 - DNA, 54 bp, Artificial
  Synthetic
attttgcaacttactactgtcaacatagtcacagtacccatcccacagtgttac

SEQ ID NO: 119 - DNA, 54 bp, Artificial
  Synthetic
gtaacactgtgggatgggtactgtgactatgttgacagtagtaagttgcaaaat

SEQ ID NO: 120 - DNA, 41 bp, Artificial; identical to SEQ ID NO: 108
  Synthetic

SEQ ID NO: 121 - DNA, 56 bp, Artificial
  Synthetic
attttgcagtgtattactgtcaccattatggtcactcacctcccacagtgattcag

SEQ ID NO: 122 - DNA, 56 bp, Artificial
  Synthetic
ctgaatcactgtgggaggtgagtgaccataatggtgacagtaatacactgcaaaat

SEQ ID NO: 123 - DNA, 19 bp, Artificial
  Synthetic
cttactactgtcaacatag

SEQ ID NO: 124 - DNA, 19 bp, Artificial
  Synthetic
cagcagtctgcaacctgaa

SEQ ID NO: 125 - DNA, 18 bp, Artificial
  Synthetic
ggctcgtcctcacacatc

SEQ ID NO: 126 - DNA, 17 bp, Artificial
  Synthetic
tactgtcaccattatgg

SEQ ID NO: 127 - DNA, 19 bp, Artificial
  Synthetic
gcagactggagcctgaaga

SEQ ID NO: 128 - DNA, 23 bp, Artificial
  Synthetic
aagctgaatcactgtgggaggtg

SEQ ID NO: 129 - DNA, 22 bp, Artificial
  Synthetic
aagaagcacacgactgaggcac

SEQ ID NO: 130 - DNA, 22 bp, Artificial
  Synthetic
ggaagatggatacagttggtgc

SEQ ID NO: 131 - protein, 95 aa, Artificial
  Synthetic
EIVLTQSPGTLSLSPGERATLSCRASQSVSSSYLAWYQQKPGQAPRLLIYGASSRATGIPDRFSGSGSGTDFTLTISRLEPEDFAVYYCHHYGHS

SEQ ID NO: 132 - protein, 96 aa, Artificial
  Synthetic
EIVLTQSPGTLSLSPGERATLSCRASQSVSSSYLAWYQQKPGQAPRLLIYGASSRATGIPDRFSGSGSGTDFTLTISRLEPEDFAVYYCQQYGSSP

SEQ ID NO: 133 - protein, 95 aa, Artificial
  Synthetic
DIQMTQSPSSLSASVGDRVTITCRASQSISSYLNWYQQKPGKAPKLLIYAASSLQSGVPSRFSGSGSGTDFTLTISSLQPEDFATYYCQHSHSTH

SEQ ID NO: 134 - protein, 95 aa, Artificial; identical to SEQ ID NO: 1
  Synthetic

SEQ ID NO: 135 - protein, 95 aa, Artificial
  Synthetic
DIQMTQSPSSLSASVGDRVTITCRASQSISSYLNWYQQKPGKAPKLLIYAASSLQSGVPSRFSGSGSGTDFTLTISSLQPEDFATYYCQHSHSTK

SEQ ID NO: 136 - protein, 108 aa, Artificial
  Synthetic
DIQMTQSPSSLSASVGDRVTFTCRTSHSISSYLNWYQQKPGKAPKILIYAVSSLYTGVPSRFSASGSGTDFTLTISSLQPEDFATYTCQQSYNIPFTFGPGTKVDIKR

SEQ ID NO: 137 - protein, 103 aa, Artificial
  Synthetic
AIQMTQSPSSLSASVGDRVTITCRASQIISNFLNWYQQKPGKAPKLLIYGAYNLQSGVPSRFSGSGSGTDFTLTISSLQPEDFAIYYCQHLTFGGGTKVEIKR

SEQ ID NO: 138 - protein, 109 aa, Artificial
  Synthetic
DIQMTQSPSSLSASVGDRVTITCRASHNINNYLNWYHQKPGKAPNLLIYAASSLQSGVPSRFSGSGSGTDYTLTISTLHPEDFGNYYCQQSYSTSMYTFGQGTQLEIKR

SEQ ID NO: 139 - protein, 108 aa, Artificial
  Synthetic
DIQMTQSPSSLSASVGDRVTITCRASQSISSYLNWYQQKPGKAPKLLIYAASSLQSGVPSRFSGSGSGTDFTLTISSLQPEDFATYHCQQSYSIPITFGQGTRLEIKR

SEQ ID NO: 140 - protein, 108 aa, Artificial
  Synthetic
DIQMTQSPSSLSASVGDRVTIACRASQTISSNLNWYQQKPGKAPKLLIYAASSLQSGVPSRFSGSGSGTDFTLTISSLQPEDFATYYCHQSYITPITFGQGTRLEIKR

SEQ ID NO: 141 - protein, 108 aa, Artificial
  Synthetic
DIQMTQSPSSLSASVGDRVTITCRASQSISSYLNWYQQKPGKAPNLLIYDASSLQSGVPSRFSGSGSGTDFTLTITSLHPEDFATYYCQQSHSTPITFGQGTRLEIKR

SEQ ID NO: 142 - protein, 108 aa, Artificial
  Synthetic
AIQLTQSPSSLSASVGDRVTITCRASQSISSYLNWYQQKPGKAPNLLIYDASSLQSGVPSRFSGSGSGTDFTLTITSLQPEDFATYYCQQSHSTPITFGQGTRLEIKR

SEQ ID NO: 143 - protein, 109 aa, Artificial
  Synthetic
AIQMTQSPSSLSASVGDRVTITCRASQNINSYLHWYQQKPGKAPKLLIYDASSFQSGVPSRFSGSGSGTDFTLTISSLQPEDFATYYCQQSYSTPPITFGQGTRVEIKR

SEQ ID NO: 144 - protein, 109 aa, Artificial
  Synthetic
AIQLTQSPSSLSASVGDRVTITCRASQSISSYLNWYQQKPGKAPKLLIYAASSLQSGVPSRFSGSKSGTDFTLTISSLQPEDFATYYCQQSYSIHPITFGQGTKLEIKR

SEQ ID NO: 145 - protein, 108 aa, Artificial
  Synthetic
AIQMTQSPSSLSASVGDRVTITCRASQSISSYLNWYQQKPGKAPKLLIYAASSLQSGVPSRFSGSGSGTDFTLTISSLQPEDFATYYCQQSHSIPPITFGQGTRLEIK

SEQ ID NO: 146 - protein, 109 aa, Artificial
  Synthetic
AIQLTQSPSSLSASVGDRVTITCRASQSISSYLNWYQQKPGKAPKLLMYAASSLQSGVPSRFSGTGSGTDFTLTISSLQREDFATYYCQQSHSTPPITFGQGTKVEIKR